European Patent Specification EP 3 761 989 B1, published May 13, 2026. Title: IMIDAZODIAZEPINEDIONES AND METHODS OF USE THEREOF. Applicant: GOLDFINCH BIO, INC. Application PCT/US2019/020732. The sequence listing filed with the application follows.

SEQUENCE LISTING (1 sequence)

SEQ ID NO: 1 - DNA, 8541 bp, Artificial Sequence
  Description of Artificial Sequence: Synthetic polynucleotide
gacggatcgggagatctcccgatcccctatggtgcactctcagtacaatctgctctgatgccgcatagttaagccagtatctgctccctgcttgtgtgttggaggtcgctgagtagtgcgcgagcaaaatttaagctacaacaaggcaaggcttgaccgacaattgcatgaagaatctgcttagggttaggcgttttgcgctgcttcgcgatgtacgggccagatatacgcgttgacattgattattgactagttattaatagtaatcaattacggggtcattagttcatagcccatatatggagttccgcgttacataacttacggtaaatggcccgcctggctgaccgcccaacgacccccgcccattgacgtcaataatgacgtatgttcccatagtaacgccaatagggactttccattgacgtcaatgggtggagtatttacggtaaactgcccacttggcagtacatcaagtgtatcatatgccaagtacgccccctattgacgtcaatgacggtaaatggcccgcctggcattatgcccagtacatgaccttatgggactttcctacttggcagtacatctacgtattagtcatcgctattaccatggtgatgcggttttggcagtacatcaatgggcgtggatagcggtttgactcacggggatttccaagtctccaccccattgacgtcaatgggagtttgttttggcaccaaaatcaacgggactttccaaaatgtcgtaacaactccgccccattgacgcaaatgggcggtaggcgtgtacggtgggaggtctatataagcagagctctccctatcagtgatagagatctccctatcagtgatagagatcgtcgacgagctcgtttagtgaaccgtcagatcgcctggagacgccatccacgctgttttgacctccatagaagacaccgggaccgatccagcctccggactctagcgtttaaacttaagcccaagctggctagaccgccatggcccaactgtactacaaaaaggtcaactactcaccgtacagagaccgcatccccctgcaaattgtgagggctgagacagagctctctgcagaggagaaggccttcctcaatgctgtggagaagggggactatgccactgtgaagcaggcccttcaggaggctgagatctactataatgttaacatcaactgcatggaccccttgggccggagtgccctgctcattgccattgagaacgagaacctggagatcatggagctactgctgaaccacagcgtgtatgtgggtgatgcattgctctatgccatacgcaaggaagtggtgggcgctgtggagcttctgctcagctacaggcggcccagcggagagaagcaggtccccactctgatgatggacacgcagttctctgaattcacaccggacatcactcccatcatgctggctgcccacaccaacaactacgaaatcatcaaactgcttgtccaaaaacgggtcactatcccacggccccaccagatccgctgcaactgtgtggagtgtgtgtctagttcagaggtagacagcctgcgccactctcgctcccgactgaacatctataaggctctggcaagcccctcactcattgccttatcaagtgaggaccccatcctaactgccttccgtctgggctgggagctcaaggagctcagcaaggtggagaatgagttcaaggccgagtatgaggagctctctcagcagtgcaagctctttgccaaagacctgctggaccaagctcggagctccagggaactggagatcatcctcaaccatcgagatgaccacagtgaagagcttgaccctcagaagtaccatgacctggccaagttgaaggtggcaatcaaataccaccagaaagagtttgttgctcagcccaactgccaacagttgcttgccaccctgtggtatgatggcttccctggatggcggcggaaacactgggtagtcaagcttctaacctgcatgaccattgggttcctgtttcccatgctgtctatagcctacctgatctcacccaggagcaaccttgggctgttcatcaagaaaccctttatcaagtttatctgccacacagcatcctatttgaccttcctctttatgcttctcctggcttctcagcacattgtcaggacagaccttcatgtacaggggcctcccccaactgtcgtggaatggatgatattgccttgggttctaggtttcatttggggtgagattaaggaaatgtgggatggtggatttactgaatacatccatgactggtggaacctgatggattttgcaatgaactccctctacctggcaactatttccctgaagattgtggcctatgtcaagtataatggttctcgtccaagggaggaatgggaaatgtggcacccgactctgattgcggaagcactcttcgcaatatccaacattttaagttcgttgcgtctcatatccctgttcacagccaactcccacttaggacctctgcagatctctttgggacgcatgctgcttgatatcctcaaattcctctttatctactgcctggtactactagcttttgccaatggactgaaccagctttacttctattatgaaaccagagctatcgatgagcctaacaactgcaaggggatccgatgtgagaaacagaacaatgccttctccacgctctttgagactcttcagtcactcttctggtctgtatttggccttttaaatctatatgtcaccaatgtgaaagccagacacgaattcaccgagtttgtaggagctaccatgtttggaacatacaatgtcatctccctggtagtgctgctgaacatgctgattgctatgatgaacaactcctatcagcttattgccgatcatgctgatatcgagtggaagtttgcaaggacgaagctctggatgagttactttgatgaaggtggcaccttgccacctcctttcaacatcatccccagccccaagtcatttctataccttggtaactggttcaacaacaccttctgccccaaaagagaccctgacggtagacggagaaggcgcaacttgagaagtttcacagaacgcaatgctgacagcctgatacaaaatcaacattatcaggaagttatcaggaatttagtcaaaagatatgtggctgctatgataagaaattccaaaacacatgagggacttacagaagaaaattttaaggaattaaagcaagacatctccagctttcggtatgaagtgcttgacctcttgggaaatagaaaacatccaaggagcttttccactagcagcactgaactgtctcagagagacgataataatgatggcagtggtggggctcgggccaaatccaagagtgtctcttttaatttaggctgcaagaaaaagacttgccatgggccacctctcatcagaaccatgccaaggtccagtggtgcccaaggaaagtcaaaagctgagtcatcaagcaaacgctccttcatgggtccttctctcaagaaactgggtctcctattctccaaatttaatggtcatatgtctgaacccagttcagagccaatgtacacaatttctgatggaattgttcagcagcactgtatgtggcaggacatcagatattctcagatggagaaagggaaagcagaggcctgttctcaaagtgaaattaacctcagtgaggtagaattaggtgaagtccagggcgctgctcagagcagtgaatgccctctagcctgttccagctctcttcactgtgcatccagcatctgctcctcaaattctaaacttttagactcctcagaggatgtatttgaaacttggggagaggcttgtgacttgctcatgcacaaatggggtgatggacaggaagaacaagttacaactcgcctctaatgactcgagtctagagggcccgtttaaacccgctgatcagcctcgactgtgccttctagttgccagccatctgttgtttgcccctcccccgtgccttccttgaccctggaaggtgccactcccactgtcctttcctaataaaatgaggaaattgcatcgcattgtctgagtaggtgtcattctattctggggggtggggtggggcaggacagcaagggggaggattgggaagacaatagcaggcatgctggggatgcggtgggctctatggcttctgaggcggaaagaaccagctggggctctagggggtatccccacgcgccctgtagcggcgcattaagcgcggcgggtgtggtggttacgcgcagcgtgaccgctacacttgccagcgccctagcgcccgctcctttcgctttcttcccttcctttctcgccacgttcgccggctttccccgtcaagctctaaatcgggggctccctttagggttccgatttagtgctttacggcacctcgaccccaaaaaacttgattagggtgatggttcacgtagtgggccatcgccctgatagacggtttttcgccctttgacgttggagtccacgttctttaatagtggactcttgttccaaactggaacaacactcaaccctatctcggtctattcttttgatttataagggattttgccgatttcggcctattggttaaaaaatgagctgatttaacaaaaatttaacgcgaattaattctgtggaatgtgtgtcagttagggtgtggaaagtccccaggctccccagcaggcagaagtatgcaaagcatgcatctcaattagtcagcaaccaggtgtggaaagtccccaggctccccagcaggcagaagtatgcaaagcatgcatctcaattagtcagcaaccatagtcccgcccctaactccgcccatcccgcccctaactccgcccagttccgcccattctccgccccatggctgactaattttttttatttatgcagaggccgaggccgcctctgcctctgagctattccagaagtagtgaggaggcttttttggaggcctaggcttttgcaaaaagctcccgggagcttgtatatccattttcggatctgatcagcacgtgatgaaaaagcctgaactcaccgcgacgtctgtcgagaagtttctgatcgaaaagttcgacagcgtctccgacctgatgcagctctcggagggcgaagaatctcgtgctttcagcttcgatgtaggagggcgtggatatgtcctgcgggtaaatagctgcgccgatggtttctacaaagatcgttatgtttatcggcactttgcatcggccgcgctcccgattccggaagtgcttgacattggggaattcagcgagagcctgacctattgcatctcccgccgtgcacagggtgtcacgttgcaagacctgcctgaaaccgaactgcccgctgttctgcagccggtcgcggaggccatggatgcgatcgctgcggccgatcttagccagacgagcgggttcggcccattcggaccgcaaggaatcggtcaatacactacatggcgtgatttcatatgcgcgattgctgatccccatgtgtatcactggcaaactgtgatggacgacaccgtcagtgcgtccgtcgcgcaggctctcgatgagctgatgctttgggccgaggactgccccgaagtccggcacctcgtgcacgcggatttcggctccaacaatgtcctgacggacaatggccgcataacagcggtcattgactggagcgaggcgatgttcggggattcccaatacgaggtcgccaacatcttcttctggaggccgtggttggcttgtatggagcagcagacgcgctacttcgagcggaggcatccggagcttgcaggatcgccgcggctccgggcgtatatgctccgcattggtcttgaccaactctatcagagcttggttgacggcaatttcgatgatgcagcttgggcgcagggtcgatgcgacgcaatcgtccgatccggagccgggactgtcgggcgtacacaaatcgcccgcagaagcgcggccgtctggaccgatggctgtgtagaagtactcgccgatagtggaaaccgacgccccagcactcgtccgagggcaaaggaatagcacgtgctacgagatttcgattccaccgccgccttctatgaaaggttgggcttcggaatcgttttccgggacgccggctggatgatcctccagcgcggggatctcatgctggagttcttcgcccaccccaacttgtttattgcagcttataatggttacaaataaagcaatagcatcacaaatttcacaaataaagcatttttttcactgcattctagttgtggtttgtccaaactcatcaatgtatcttatcatgtctgtataccgtcgacctctagctagagcttggcgtaatcatggtcatagctgtttcctgtgtgaaattgttatccgctcacaattccacacaacatacgagccggaagcataaagtgtaaagcctggggtgcctaatgagtgagctaactcacattaattgcgttgcgctcactgcccgctttccagtcgggaaacctgtcgtgccagctgcattaatgaatcggccaacgcgcggggagaggcggtttgcgtattgggcgctcttccgcttcctcgctcactgactcgctgcgctcggtcgttcggctgcggcgagcggtatcagctcactcaaaggcggtaatacggttatccacagaatcaggggataacgcaggaaagaacatgtgagcaaaaggccagcaaaaggccaggaaccgtaaaaaggccgcgttgctggcgtttttccataggctccgcccccctgacgagcatcacaaaaatcgacgctcaagtcagaggtggcgaaacccgacaggactataaagataccaggcgtttccccctggaagctccctcgtgcgctctcctgttccgaccctgccgcttaccggatacctgtccgcctttctcccttcgggaagcgtggcgctttctcatagctcacgctgtaggtatctcagttcggtgtaggtcgttcgctccaagctgggctgtgtgcacgaaccccccgttcagcccgaccgctgcgccttatccggtaactatcgtcttgagtccaacccggtaagacacgacttatcgccactggcagcagccactggtaacaggattagcagagcgaggtatgtaggcggtgctacagagttcttgaagtggtggcctaactacggctacactagaagaacagtatttggtatctgcgctctgctgaagccagttaccttcggaaaaagagttggtagctcttgatccggcaaacaaaccaccgctggtagcggttggttttttgtttgcaagcagcagattacgcgcagaaaaaaaggatctcaagaagatcctttgatcttttctacggggtctgacgctcagtggaacgaaaactcacgttaagggattttggtcatgagattatcaaaaaggatcttcacctagatccttttaaattaaaaatgaagttttaaatcaatctaaagtatatatgagtaaacttggtctgacagttaccaatgcttaatcagtgaggcacctatctcagcgatctgtctatttcgttcatccatagttgcctgactccccgtcgtgtagataactacgatacgggagggcttaccatctggccccagtgctgcaatgataccgcgagacccacgctcaccggctccagatttatcagcaataaaccagccagccggaagggccgagcgcagaagtggtcctgcaactttatccgcctccatccagtctattaattgttgccgggaagctagagtaagtagttcgccagttaatagtttgcgcaacgttgttgccattgctacaggcatcgtggtgtcacgctcgtcgtttggtatggcttcattcagctccggttcccaacgatcaaggcgagttacatgatcccccatgttgtgcaaaaaagcggttagctccttcggtcctccgatcgttgtcagaagtaagttggccgcagtgttatcactcatggttatggcagcactgcataattctcttactgtcatgccatccgtaagatgcttttctgtgactggtgagtactcaaccaagtcattctgagaatagtgtatgcggcgaccgagttgctcttgcccggcgtcaatacgggataataccgcgccacatagcagaactttaaaagtgctcatcattggaaaacgttcttcggggcgaaaactctcaaggatcttaccgctgttgagatccagttcgatgtaacccactcgtgcacccaactgatcttcagcatcttttactttcaccagcgtttctgggtgagcaaaaacaggaaggcaaaatgccgcaaaaaagggaataagggcgacacggaaatgttgaatactcatactcttcctttttcaatattattgaagcatttatcagggttattgtctcatgagcggatacatatttgaatgtatttagaaaaataaacaaataggggttccgcgcacatttccccgaaaagtgccacctgacgtc